European Patent Application EP 4 553 500 A1, published May 14, 2025. Title: Verfahren zum Nachweis und zur Bestimmung der Bindungsstärke wenigstens eines Analyten in einer Probe. Applicant: attomolMolekulare Diagnostika GmbH. Application EP. The sequence listing filed with the application follows.

SEQUENCE LISTING (5 sequences)

SEQ ID NO: 1 - protein, 39 aa, synthetic construct
PTTTTTTTTTTTTTTTTTGATACTCTCGTACCTTGAGTG

SEQ ID NO: 2 - protein, 80 aa, synthetic construct
GATCTGCACTGTACTAGTACACTCAAGGTACGAGAGTATCACTGCGTTGCGTATATTTCGTTGCGAACGCAGTACTAGTC

SEQ ID NO: 3 - protein, 20 aa, synthetic construct
GTTGCGTATATTTCGTTGCG

SEQ ID NO: 4 - protein, 30 aa, synthetic construct
CTAGTACAGTGCAGATCGACTAGTACTGCG

SEQ ID NO: 5 - protein, 23 aa, synthetic construct
GCSHQESTCITGRSCITGRSGRC